European Patent Application EP 4 339 281 A1, published March 20, 2024. Title: Geranylgeranyl pyrophosphate synthase variant and method of producing tetraterpene, precursor thereof and compounds in which the precursor is tetraterpene using the variant. Applicant: CJ CheilJedang Corporation. The sequence listing filed with the application follows.

SEQUENCE LISTING (91 sequences)

SEQ ID NO: 1 - protein, 327 aa, Artificial Sequence
  GGS1_WT
MDYNSADFKEIWGKAADTALLGPYNYLANNRGHNIREHLIAAFGAVIKVDKSDLETISHITKILHNSSLLVDDVEDNSMLRRGLPAAHCLFGVPQTINSANYMYFVALQEVLKLKSYDAVSIFTEEMINLHRGQGMDLYWRETLTCPSEDEYLEMVVHKTGGLFRLALRLMLSVASKQEDHEKINFDLTHLTDTLGVIYQILDDYLNLQSTELTENKGFCEDISEGKFSFPLIHSIRTNPDNHEILNILKQRTSDASLKKYAVDYMRTETKSFDYCLKRIQAMSLKASSYIDDLAAAGHDVSKLRAILHYFVSTSDCEERKYFEDAQ

SEQ ID NO: 2 - DNA, 984 bp, Artificial Sequence
  ggs1_WT
atggattataacagcgcggatttcaaggagatatggggcaaggccgccgacaccgcgctgctgggaccgtacaactacctcgccaacaaccggggccacaacatcagagaacacttgatcgcagcgttcggagcggttatcaaggtggacaagagcgatctcgagaccatttcgcacatcaccaagattttgcataactcgtcgctgcttgttgatgacgtggaagacaactcgatgctccgacgaggcctgccggcagcccattgtctgtttggagtcccccaaaccatcaactccgccaactacatgtactttgtggctctgcaggaggtgctcaagctcaagtcttatgatgccgtctccattttcaccgaggaaatgatcaacttgcatagaggtcagggtatggatctctactggagagaaacactcacttgcccctcggaagacgagtatctggagatggtggtgcacaagaccggtggactgtttcggctggctctgagacttatgctgtcggtggcatcgaaacaggaggaccatgaaaagatcaactttgatctcacacaccttaccgacacactgggagtcatttaccagattctggatgattacctcaacctgcagtccacggaattgaccgagaacaagggattctgcgaagatatcagcgaaggaaagttttcgtttccgctgattcacagcatacgcaccaacccggataaccacgagattctcaacattctcaaacagcgaacaagcgacgcttcactcaaaaagtacgccgtggactacatgagaacagaaaccaagagtttcgactactgcctcaagaggatacaggccatgtcactcaaggcaagttcgtacattgatgatctagcagcagctggccacgatgtctccaagctacgagccattttgcattattttgtgtccacctctgactgtgaggagagaaagtactttgaggatgcgcagtga

SEQ ID NO: 3 - protein, 327 aa, Artificial Sequence
  GGS1_M103I
MDYNSADFKEIWGKAADTALLGPYNYLANNRGHNIREHLIAAFGAVIKVDKSDLETISHITKILHNSSLLVDDVEDNSMLRRGLPAAHCLFGVPQTINSANYIYFVALQEVLKLKSYDAVSIFTEEMINLHRGQGMDLYWRETLTCPSEDEYLEMVVHKTGGLFRLALRLMLSVASKQEDHEKINFDLTHLTDTLGVIYQILDDYLNLQSTELTENKGFCEDISEGKFSFPLIHSIRTNPDNHEILNILKQRTSDASLKKYAVDYMRTETKSFDYCLKRIQAMSLKASSYIDDLAAAGHDVSKLRAILHYFVSTSDCEERKYFEDAQ

SEQ ID NO: 4 - DNA, 984 bp, Artificial Sequence
  ggs1_G309A
atggattataacagcgcggatttcaaggagatatggggcaaggccgccgacaccgcgctgctgggaccgtacaactacctcgccaacaaccggggccacaacatcagagaacacttgatcgcagcgttcggagcggttatcaaggtggacaagagcgatctcgagaccatttcgcacatcaccaagattttgcataactcgtcgctgcttgttgatgacgtggaagacaactcgatgctccgacgaggcctgccggcagcccattgtctgtttggagtcccccaaaccatcaactccgccaactacatatactttgtggctctgcaggaggtgctcaagctcaagtcttatgatgccgtctccattttcaccgaggaaatgatcaacttgcatagaggtcagggtatggatctctactggagagaaacactcacttgcccctcggaagacgagtatctggagatggtggtgcacaagaccggtggactgtttcggctggctctgagacttatgctgtcggtggcatcgaaacaggaggaccatgaaaagatcaactttgatctcacacaccttaccgacacactgggagtcatttaccagattctggatgattacctcaacctgcagtccacggaattgaccgagaacaagggattctgcgaagatatcagcgaaggaaagttttcgtttccgctgattcacagcatacgcaccaacccggataaccacgagattctcaacattctcaaacagcgaacaagcgacgcttcactcaaaaagtacgccgtggactacatgagaacagaaaccaagagtttcgactactgcctcaagaggatacaggccatgtcactcaaggcaagttcgtacattgatgatctagcagcagctggccacgatgtctccaagctacgagccattttgcattattttgtgtccacctctgactgtgaggagagaaagtactttgaggatgcgcagtga

SEQ ID NO: 5 - protein, 327 aa, Artificial Sequence
  GGS1_F43I
MDYNSADFKEIWGKAADTALLGPYNYLANNRGHNIREHLIAAIGAVIKVDKSDLETISHITKILHNSSLLVDDVEDNSMLRRGLPAAHCLFGVPQTINSANYMYFVALQEVLKLKSYDAVSIFTEEMINLHRGQGMDLYWRETLTCPSEDEYLEMVVHKTGGLFRLALRLMLSVASKQEDHEKINFDLTHLTDTLGVIYQILDDYLNLQSTELTENKGFCEDISEGKFSFPLIHSIRTNPDNHEILNILKQRTSDASLKKYAVDYMRTETKSFDYCLKRIQAMSLKASSYIDDLAAAGHDVSKLRAILHYFVSTSDCEERKYFEDAQ

SEQ ID NO: 6 - DNA, 984 bp, Artificial Sequence
  ggs1_T127A
atggattataacagcgcggatttcaaggagatatggggcaaggccgccgacaccgcgctgctgggaccgtacaactacctcgccaacaaccggggccacaacatcagagaacacttgatcgcagcgatcggagcggttatcaaggtggacaagagcgatctcgagaccatttcgcacatcaccaagattttgcataactcgtcgctgcttgttgatgacgtggaagacaactcgatgctccgacgaggcctgccggcagcccattgtctgtttggagtcccccaaaccatcaactccgccaactacatgtactttgtggctctgcaggaggtgctcaagctcaagtcttatgatgccgtctccattttcaccgaggaaatgatcaacttgcatagaggtcagggtatggatctctactggagagaaacactcacttgcccctcggaagacgagtatctggagatggtggtgcacaagaccggtggactgtttcggctggctctgagacttatgctgtcggtggcatcgaaacaggaggaccatgaaaagatcaactttgatctcacacaccttaccgacacactgggagtcatttaccagattctggatgattacctcaacctgcagtccacggaattgaccgagaacaagggattctgcgaagatatcagcgaaggaaagttttcgtttccgctgattcacagcatacgcaccaacccggataaccacgagattctcaacattctcaaacagcgaacaagcgacgcttcactcaaaaagtacgccgtggactacatgagaacagaaaccaagagtttcgactactgcctcaagaggatacaggccatgtcactcaaggcaagttcgtacattgatgatctagcagcagctggccacgatgtctccaagctacgagccattttgcattattttgtgtccacctctgactgtgaggagagaaagtactttgaggatgcgcagtga

SEQ ID NO: 7 - protein, 327 aa, Artificial Sequence
  GGS1_N29T/L90R
MDYNSADFKEIWGKAADTALLGPYNYLATNRGHNIREHLIAAFGAVIKVDKSDLETISHITKILHNSSLLVDDVEDNSMLRRGLPAAHCRFGVPQTINSANYMYFVALQEVLKLKSYDAVSIFTEEMINLHRGQGMDLYWRETLTCPSEDEYLEMVVHKTGGLFRLALRLMLSVASKQEDHEKINFDLTHLTDTLGVIYQILDDYLNLQSTELTENKGFCEDISEGKFSFPLIHSIRTNPDNHEILNILKQRTSDASLKKYAVDYMRTETKSFDYCLKRIQAMSLKASSYIDDLAAAGHDVSKLRAILHYFVSTSDCEERKYFEDAQ

SEQ ID NO: 8 - DNA, 984 bp, Artificial Sequence
  ggs1_A86C_T269G
atggattataacagcgcggatttcaaggagatatggggcaaggccgccgacaccgcgctgctgggaccgtacaactacctcgccaccaaccggggccacaacatcagagaacacttgatcgcagcgttcggagcggttatcaaggtggacaagagcgatctcgagaccatttcgcacatcaccaagattttgcataactcgtcgctgcttgttgatgacgtggaagacaactcgatgctccgacgaggcctgccggcagcccattgtcggtttggagtcccccaaaccatcaactccgccaactacatgtactttgtggctctgcaggaggtgctcaagctcaagtcttatgatgccgtctccattttcaccgaggaaatgatcaacttgcatagaggtcagggtatggatctctactggagagaaacactcacttgcccctcggaagacgagtatctggagatggtggtgcacaagaccggtggactgtttcggctggctctgagacttatgctgtcggtggcatcgaaacaggaggaccatgaaaagatcaactttgatctcacacaccttaccgacacactgggagtcatttaccagattctggatgattacctcaacctgcagtccacggaattgaccgagaacaagggattctgcgaagatatcagcgaaggaaagttttcgtttccgctgattcacagcatacgcaccaacccggataaccacgagattctcaacattctcaaacagcgaacaagcgacgcttcactcaaaaagtacgccgtggactacatgagaacagaaaccaagagtttcgactactgcctcaagaggatacaggccatgtcactcaaggcaagttcgtacattgatgatctagcagcagctggccacgatgtctccaagctacgagccattttgcattattttgtgtccacctctgactgtgaggagagaaagtactttgaggatgcgcagtga

SEQ ID NO: 9 - protein, 327 aa, Artificial Sequence
  GGS1_N29T
MDYNSADFKEIWGKAADTALLGPYNYLATNRGHNIREHLIAAFGAVIKVDKSDLETISHITKILHNSSLLVDDVEDNSMLRRGLPAAHCLFGVPQTINSANYMYFVALQEVLKLKSYDAVSIFTEEMINLHRGQGMDLYWRETLTCPSEDEYLEMVVHKTGGLFRLALRLMLSVASKQEDHEKINFDLTHLTDTLGVIYQILDDYLNLQSTELTENKGFCEDISEGKFSFPLIHSIRTNPDNHEILNILKQRTSDASLKKYAVDYMRTETKSFDYCLKRIQAMSLKASSYIDDLAAAGHDVSKLRAILHYFVSTSDCEERKYFEDAQ

SEQ ID NO: 10 - DNA, 984 bp, Artificial Sequence
  ggs1_A86C
atggattataacagcgcggatttcaaggagatatggggcaaggccgccgacaccgcgctgctgggaccgtacaactacctcgccaccaaccggggccacaacatcagagaacacttgatcgcagcgttcggagcggttatcaaggtggacaagagcgatctcgagaccatttcgcacatcaccaagattttgcataactcgtcgctgcttgttgatgacgtggaagacaactcgatgctccgacgaggcctgccggcagcccattgtctgtttggagtcccccaaaccatcaactccgccaactacatgtactttgtggctctgcaggaggtgctcaagctcaagtcttatgatgccgtctccattttcaccgaggaaatgatcaacttgcatagaggtcagggtatggatctctactggagagaaacactcacttgcccctcggaagacgagtatctggagatggtggtgcacaagaccggtggactgtttcggctggctctgagacttatgctgtcggtggcatcgaaacaggaggaccatgaaaagatcaactttgatctcacacaccttaccgacacactgggagtcatttaccagattctggatgattacctcaacctgcagtccacggaattgaccgagaacaagggattctgcgaagatatcagcgaaggaaagttttcgtttccgctgattcacagcatacgcaccaacccggataaccacgagattctcaacattctcaaacagcgaacaagcgacgcttcactcaaaaagtacgccgtggactacatgagaacagaaaccaagagtttcgactactgcctcaagaggatacaggccatgtcactcaaggcaagttcgtacattgatgatctagcagcagctggccacgatgtctccaagctacgagccattttgcattattttgtgtccacctctgactgtgaggagagaaagtactttgaggatgcgcagtga

SEQ ID NO: 11 - protein, 327 aa, Artificial Sequence
  GGS1_L90R
MDYNSADFKEIWGKAADTALLGPYNYLANNRGHNIREHLIAAFGAVIKVDKSDLETISHITKILHNSSLLVDDVEDNSMLRRGLPAAHCRFGVPQTINSANYMYFVALQEVLKLKSYDAVSIFTEEMINLHRGQGMDLYWRETLTCPSEDEYLEMVVHKTGGLFRLALRLMLSVASKQEDHEKINFDLTHLTDTLGVIYQILDDYLNLQSTELTENKGFCEDISEGKFSFPLIHSIRTNPDNHEILNILKQRTSDASLKKYAVDYMRTETKSFDYCLKRIQAMSLKASSYIDDLAAAGHDVSKLRAILHYFVSTSDCEERKYFEDAQ

SEQ ID NO: 12 - DNA, 984 bp, Artificial Sequence
  ggs1_T269G
atggattataacagcgcggatttcaaggagatatggggcaaggccgccgacaccgcgctgctgggaccgtacaactacctcgccaacaaccggggccacaacatcagagaacacttgatcgcagcgttcggagcggttatcaaggtggacaagagcgatctcgagaccatttcgcacatcaccaagattttgcataactcgtcgctgcttgttgatgacgtggaagacaactcgatgctccgacgaggcctgccggcagcccattgtcggtttggagtcccccaaaccatcaactccgccaactacatgtactttgtggctctgcaggaggtgctcaagctcaagtcttatgatgccgtctccattttcaccgaggaaatgatcaacttgcatagaggtcagggtatggatctctactggagagaaacactcacttgcccctcggaagacgagtatctggagatggtggtgcacaagaccggtggactgtttcggctggctctgagacttatgctgtcggtggcatcgaaacaggaggaccatgaaaagatcaactttgatctcacacaccttaccgacacactgggagtcatttaccagattctggatgattacctcaacctgcagtccacggaattgaccgagaacaagggattctgcgaagatatcagcgaaggaaagttttcgtttccgctgattcacagcatacgcaccaacccggataaccacgagattctcaacattctcaaacagcgaacaagcgacgcttcactcaaaaagtacgccgtggactacatgagaacagaaaccaagagtttcgactactgcctcaagaggatacaggccatgtcactcaaggcaagttcgtacattgatgatctagcagcagctggccacgatgtctccaagctacgagccattttgcattattttgtgtccacctctgactgtgaggagagaaagtactttgaggatgcgcagtga

SEQ ID NO: 13 - protein, 327 aa, Artificial Sequence
  GGS1_I122V/R141K
MDYNSADFKEIWGKAADTALLGPYNYLANNRGHNIREHLIAAFGAVIKVDKSDLETISHITKILHNSSLLVDDVEDNSMLRRGLPAAHCLFGVPQTINSANYMYFVALQEVLKLKSYDAVSVFTEEMINLHRGQGMDLYWKETLTCPSEDEYLEMVVHKTGGLFRLALRLMLSVASKQEDHEKINFDLTHLTDTLGVIYQILDDYLNLQSTELTENKGFCEDISEGKFSFPLIHSIRTNPDNHEILNILKQRTSDASLKKYAVDYMRTETKSFDYCLKRIQAMSLKASSYIDDLAAAGHDVSKLRAILHYFVSTSDCEERKYFEDAQ

SEQ ID NO: 14 - DNA, 984 bp, Artificial Sequence
  ggs1_A364G_G422A
atggattataacagcgcggatttcaaggagatatggggcaaggccgccgacaccgcgctgctgggaccgtacaactacctcgccaacaaccggggccacaacatcagagaacacttgatcgcagcgttcggagcggttatcaaggtggacaagagcgatctcgagaccatttcgcacatcaccaagattttgcataactcgtcgctgcttgttgatgacgtggaagacaactcgatgctccgacgaggcctgccggcagcccattgtctgtttggagtcccccaaaccatcaactccgccaactacatgtactttgtggctctgcaggaggtgctcaagctcaagtcttatgatgccgtctccgttttcaccgaggaaatgatcaacttgcatagaggtcagggtatggatctctactggaaagaaacactcacttgcccctcggaagacgagtatctggagatggtggtgcacaagaccggtggactgtttcggctggctctgagacttatgctgtcggtggcatcgaaacaggaggaccatgaaaagatcaactttgatctcacacaccttaccgacacactgggagtcatttaccagattctggatgattacctcaacctgcagtccacggaattgaccgagaacaagggattctgcgaagatatcagcgaaggaaagttttcgtttccgctgattcacagcatacgcaccaacccggataaccacgagattctcaacattctcaaacagcgaacaagcgacgcttcactcaaaaagtacgccgtggactacatgagaacagaaaccaagagtttcgactactgcctcaagaggatacaggccatgtcactcaaggcaagttcgtacattgatgatctagcagcagctggccacgatgtctccaagctacgagccattttgcattattttgtgtccacctctgactgtgaggagagaaagtactttgaggatgcgcagtga

SEQ ID NO: 15 - protein, 327 aa, Artificial Sequence
  GGS1_I122V
MDYNSADFKEIWGKAADTALLGPYNYLANNRGHNIREHLIAAFGAVIKVDKSDLETISHITKILHNSSLLVDDVEDNSMLRRGLPAAHCLFGVPQTINSANYMYFVALQEVLKLKSYDAVSVFTEEMINLHRGQGMDLYWRETLTCPSEDEYLEMVVHKTGGLFRLALRLMLSVASKQEDHEKINFDLTHLTDTLGVIYQILDDYLNLQSTELTENKGFCEDISEGKFSFPLIHSIRTNPDNHEILNILKQRTSDASLKKYAVDYMRTETKSFDYCLKRIQAMSLKASSYIDDLAAAGHDVSKLRAILHYFVSTSDCEERKYFEDAQ

SEQ ID NO: 16 - DNA, 984 bp, Artificial Sequence
  ggs1_A364G
atggattataacagcgcggatttcaaggagatatggggcaaggccgccgacaccgcgctgctgggaccgtacaactacctcgccaacaaccggggccacaacatcagagaacacttgatcgcagcgttcggagcggttatcaaggtggacaagagcgatctcgagaccatttcgcacatcaccaagattttgcataactcgtcgctgcttgttgatgacgtggaagacaactcgatgctccgacgaggcctgccggcagcccattgtctgtttggagtcccccaaaccatcaactccgccaactacatgtactttgtggctctgcaggaggtgctcaagctcaagtcttatgatgccgtctccgttttcaccgaggaaatgatcaacttgcatagaggtcagggtatggatctctactggagagaaacactcacttgcccctcggaagacgagtatctggagatggtggtgcacaagaccggtggactgtttcggctggctctgagacttatgctgtcggtggcatcgaaacaggaggaccatgaaaagatcaactttgatctcacacaccttaccgacacactgggagtcatttaccagattctggatgattacctcaacctgcagtccacggaattgaccgagaacaagggattctgcgaagatatcagcgaaggaaagttttcgtttccgctgattcacagcatacgcaccaacccggataaccacgagattctcaacattctcaaacagcgaacaagcgacgcttcactcaaaaagtacgccgtggactacatgagaacagaaaccaagagtttcgactactgcctcaagaggatacaggccatgtcactcaaggcaagttcgtacattgatgatctagcagcagctggccacgatgtctccaagctacgagccattttgcattattttgtgtccacctctgactgtgaggagagaaagtactttgaggatgcgcagtga

SEQ ID NO: 17 - protein, 327 aa, Artificial Sequence
  GGS1_R141K
MDYNSADFKEIWGKAADTALLGPYNYLANNRGHNIREHLIAAFGAVIKVDKSDLETISHITKILHNSSLLVDDVEDNSMLRRGLPAAHCLFGVPQTINSANYMYFVALQEVLKLKSYDAVSIFTEEMINLHRGQGMDLYWKETLTCPSEDEYLEMVVHKTGGLFRLALRLMLSVASKQEDHEKINFDLTHLTDTLGVIYQILDDYLNLQSTELTENKGFCEDISEGKFSFPLIHSIRTNPDNHEILNILKQRTSDASLKKYAVDYMRTETKSFDYCLKRIQAMSLKASSYIDDLAAAGHDVSKLRAILHYFVSTSDCEERKYFEDAQ

SEQ ID NO: 18 - DNA, 984 bp, Artificial Sequence
  ggs1_G422A
atggattataacagcgcggatttcaaggagatatggggcaaggccgccgacaccgcgctgctgggaccgtacaactacctcgccaacaaccggggccacaacatcagagaacacttgatcgcagcgttcggagcggttatcaaggtggacaagagcgatctcgagaccatttcgcacatcaccaagattttgcataactcgtcgctgcttgttgatgacgtggaagacaactcgatgctccgacgaggcctgccggcagcccattgtctgtttggagtcccccaaaccatcaactccgccaactacatgtactttgtggctctgcaggaggtgctcaagctcaagtcttatgatgccgtctccattttcaccgaggaaatgatcaacttgcatagaggtcagggtatggatctctactggaaagaaacactcacttgcccctcggaagacgagtatctggagatggtggtgcacaagaccggtggactgtttcggctggctctgagacttatgctgtcggtggcatcgaaacaggaggaccatgaaaagatcaactttgatctcacacaccttaccgacacactgggagtcatttaccagattctggatgattacctcaacctgcagtccacggaattgaccgagaacaagggattctgcgaagatatcagcgaaggaaagttttcgtttccgctgattcacagcatacgcaccaacccggataaccacgagattctcaacattctcaaacagcgaacaagcgacgcttcactcaaaaagtacgccgtggactacatgagaacagaaaccaagagtttcgactactgcctcaagaggatacaggccatgtcactcaaggcaagttcgtacattgatgatctagcagcagctggccacgatgtctccaagctacgagccattttgcattattttgtgtccacctctgactgtgaggagagaaagtactttgaggatgcgcagtga

SEQ ID NO: 19 - DNA, 58 bp, Artificial Sequence
  Primer
catatctacagcattaattaagcagatccaaaaggatccatggattataacagcgcgg

SEQ ID NO: 20 - DNA, 59 bp, Artificial Sequence
  Primer
gaatgtaagcgtgacataactaattacatgaggtacctcactgcgcatcctcaaagtac

SEQ ID NO: 21 - DNA, 40 bp, Artificial Sequence
  Primer
gaggccctttcgtcttcaagaattcgagtttggcgcccgt

SEQ ID NO: 22 - DNA, 60 bp, Artificial Sequence
  Primer
tgacataactaattacatgaggtaccggatccttttggatctgcttaattaatgctgtag

SEQ ID NO: 23 - DNA, 60 bp, Artificial Sequence
  Primer
ctacagcattaattaagcagatccaaaaggatccggtacctcatgtaattagttatgtca

SEQ ID NO: 24 - DNA, 55 bp, Artificial Sequence
  Primer
agtcagacagatactcgtcgcggccgcggcgcgccgcaaattaaagccttcgagc

SEQ ID NO: 25 - DNA, 55 bp, Artificial Sequence
  Primer
gctcgaaggctttaatttgcggcgcgccgcggccgcgacgagtatctgtctgact

SEQ ID NO: 26 - DNA, 40 bp, Artificial Sequence
  Primer
acgggcgccaaactcgaattcttgaagacgaaagggcctc

SEQ ID NO: 27 - DNA, 2019 bp, Artificial Sequence
  X. dendrorhous crtYB
atgacggctctcgcatattaccagatccatctgatctatactctcccaattcttggtcttctcggcctgctcacttccccgattttgacaaaatttgacatctacaaaatatcgatcctcgtatttattgcgtttagtgcaaccacaccatgggactcatggatcatcagaaatggcgcatggacatatccatcagcggagagtggccaaggcgtgtttggaacgtttctagatgttccatatgaagagtacgctttctttgtcattcaaaccgtaatcaccggcttggtctacgtcttggcaactaggcaccttctcccatctctcgcgcttcccaagactagatcgtccgccctttctctcgcgctcaaggcgctcatccctctgcccattatctacctatttaccgctcaccccagcccatcgcccgacccgctcgtgacagatcactacttctacatgcgggcactctccttactcatcaccccacctaccatgctcttggcagcattatcaggcgaatatgctttcgattggaaaagtggccgagcaaagtcaactattgcagcaatcatgatcccgacggtgtatctgatttgggtagattatgttgctgtcggtcaagactcttggtcgatcaacgatgagaagattgtagggtggaggcttggaggtgtactacccattgaggaagctatgttcttcttactgacgaatctaatgattgttctgggtctgtctgcctgcgatcatactcaggccctatacctgctacacggtcgaactatttatggcaacaaaaagatgccatcttcatttcccctcattacaccgcctgtgctctccctgttttttagcagccgaccatactcttctcagccaaaacgtgacttggaactggcagtcaagttgttggaggaaaagagccggagcttttttgttgcctcggctggatttcctagcgaagttagggagaggctggttggactatacgcattctgccgggtgactgatgatcttatcgactctcctgaagtatcttccaacccgcatgccacaattgacatggtctccgattttcttaccctactatttgggcccccgctacacccttcgcaacctgacaagatcctttcttcgcctttacttcctccttcgcacccttcccgacccacgggaatgtatcccctcccgcctcctccttcgctctcgcctgccgagctcgttcaattccttaccgaaagggttcccgttcaataccatttcgccttcaggttgctcgctaagttgcaagggctgatccctcgatacccactcgacgaactccttagaggatacaccactgatcttatctttcccttatcgacagaggcagtccaggctcggaagacgcctatcgagaccacagctgacttgctggactatggtctatgtgtagcaggctcagtcgccgagctattggtctatgtctcttgggcaagtgcaccaagtcaggtccctgccaccatagaagaaagagaagctgtgttagtggcaagccgagagatgggaactgcccttcagttggtgaacattgctagggacattaaaggggacgcaacagaagggagattttacctaccactctcattctttggtcttcgggatgaatcaaagcttgcgatcccgactgattggacggaacctcggcctcaagatttcgacaaactcctcagtctatctccttcgtccacattaccatcttcaaacgcctcagaaagcttccggttcgaatggaagacgtactcgcttccattagtcgcctacgcagaggatcttgccaaacattcttataagggaattgaccgacttcctaccgaggttcaagcgggaatgcgagcggcttgcgcgagctacctactgatcggccgagagatcaaagtcgtttggaaaggagacgtcggagagagaaggacagttgccggatggaggagagtacggaaagtcttgagtgtggtcatgagcggatgggaagggcag

SEQ ID NO: 28 - DNA, 1966 bp, Artificial Sequence
  X. dendrorhous crtI
atgggaaaagaacaagatcaggataaacccacagctatcatcgtgggatgtggtatcggtggaatcgccactgccgctcgtcttgctaaagaaggtttccaggtcacggtgttcgagaagaacgactactccggaggtcgatgctctttaatcgagcgagatggttatcgattcgatcaggggcccagtttgctgctcttgccagatctcttcaagcagacattcgaagatttgggagagaagatggaagattgggtcgatctcatcaagtgtgaacccaactatgtttgccacttccacgatgaagagactttcactctttcaaccgacatggcgttgctcaagcgggaagtcgagcgttttgaaggcaaagatggatttgatcggttcttgtcgtttatccaagaagcccacagacattacgagcttgctgtcgttcacgtcctgcagaagaacttccctggcttcgcagcattcttacggctacagttcattggccaaatcctggctcttcaccccttcgagtctatctggacaagagtttgtcgatatttcaagaccgacagattacgaagagtcttctcgtttgcagtgatgtacatgggtcaaagcccatacagtgcgcccggaacatattccttgctccaatacaccgaattgaccgagggcatctggtatccgagaggaggcttttggcaggttcctaatactcttcttcagatcgtcaagcgcaacaatccctcagccaagttcaatttcaacgctccagtttcccaggttcttctctctcctgccaaggaccgagcgactggtgttcgacttgaatccggcgaggaacatcacgccgatgttgtgattgtcaatgctgacctcgtttacgcctccgagcacttgattcctgacgatgccagaaacaagattggccaactgggtgaagtcaagagaagttggtgggctgacttagttggtggaaagaagctcaagggaagttgcagtagtttgagcttctactggagcatggaccgaatcgtggacggtctgggcggacacaatatcttcttggccgaggacttcaagggatcattcgacacaatcttcgaggagttgggtctcccagccgatccttccttttacgtgaacgttccctcgcgaatcgatccttctgccgctcccgaaggcaaagatgctatcgtcattcttgtgccgtgtggccatatcgacgcttcgaaccctcaagattacaacaagcttgttgctcgggcaaggaagtttgtgatccacacgctttccgccaagcttggacttcccgactttgaaaaaatgattgtggcagagaaggttcacgatgctccctcttgggagaaagaattcaacctcaaggacggaagcatcttgggactggctcacaactttatgcaagttcttggtttcaggccgagcaccagacatcccaagtatgacaagttgttctttgtcggggcttcgactcatcccggaactggggttcccatcgtcttggctggagccaagttaactgccaaccaagttctcgaatcctttgaccgatccccagctccagatcccaatatgtcactctccgtaccatatggaaaacctctcaaatcaaatggaacgggtatcgattctcaggtccagctgaagttcatggatttggagagatgggtataccttttggtgttgttgattggggccgtgatcgctcgatccgttggtgttcttgctttctgaagcaagacaacgatcctttcttagagttttattttagtctcttcctgtgttctctctatatacatactctgctcgtctgttctcttctcgagggttcctctttactttgtgtcagagtcatacccggtctctcaacgtccgtttgagggctagacaattgttagtctcgaaatctccatcacctcaagtctgatgttcatcatcttttttattcgtt

SEQ ID NO: 29 - DNA, 2830 bp, Artificial Sequence
  TEFINtp-crtYB-CYC1t
agagaccgggttggcggcgcatttgtgtcccaaaaaacagccccaattgccccaattgaccccaaattgacccagtagcgggcccaaccccggcgagagcccccttctccccacatatcaaacctcccccggttcccacacttgccgttaagggcgtagggtactgcagtctggaatctacgcttgttcagactttgtactagtttctttgtctggccatccgggtaacccatgccggacgcaaaatagactactgaaaatttttttgctttgtggttgggactttagccaagggtataaaagaccaccgtccccgaattacctttcctcttcttttctctctctccttgtcaactcacacccgaaatcgttaagcatttccttctgagtataagaatcattcaaaatggtgagtttcagaggcagcagcaattgccacgggctttgagcacacggccgggtgtggtcccattcccatcgacacaagacgccacgtcatccgaccagcactttttgcagtactaaccgcagacggctctcgcatattaccagatccatctgatctatactctcccaattcttggtcttctcggtctgctcacttccccgattttgacaaaatttgacatctacaaaatatcgatcctcgtatttattgcgtttagtgcaaccacaccatgggactcatggatcatcagaaatggcgcatggacatatccatcagcggagagtggccaaggcgtgtttggaacgtttctagatgttccatatgaagagtacgctttctttgtcattcaaaccgtaatcaccggcttggtctacgtcttggcaactaggcaccttctcccatctctcgcgcttcccaagactagatcgtccgccctttctctcgcgctcaaggcgctcatccctctgcccattatctacctatttaccgctcaccccagcccatcgcccgacccgctcgtgacagatcactacttctacatgcgggcactctccttactcatcaccccacctaccatgctcttggcagcattatcaggcgaatatgctttcgattggaaaagtggccgagcaaagtcaactattgcagcaatcatgatcccgacggtgtatctgatttgggtagattatgttgctgtcggtcaagactcttggtcgatcaacgatgagaagattgtagggtggaggcttggaggtgtactacccattgaggaagctatgttcttcttactgacgaatctaatgattgttctgggtctgtctgcctgcgatcatactcaggccctatacctgctacacggtcgaactatttatggcaacaaaaagatgccatcttcatttcccctcattacaccgcctgtgctctccctgttttttagcagccgaccatactcttctcagccaaaacgtgacttggaactggcagtcaagttgttggaggaaaagagccggagcttttttgttgcctcggctggatttcctagcgaagttagggagaggctggttggactatacgcattctgccgggtgactgatgatcttatcgactctcctgaagtatcttccaacccgcatgccacaattgacatggtctccgattttcttaccctactatttgggcccccgctacacccttcgcaacctgacaagatcctttcttcgcctttacttcctccttcgcacccttcccgacccacgggaatgtatcccctcccgcctcctccttcgctctcgcctgccgagctcgttcaattccttaccgaaagggttcccgttcaataccatttcgccttcaggttgctcgctaagttgcaagggctgatccctcgatacccactcgacgaactccttagaggatacaccactgatcttatctttcctttatcgacagaggcagtccaggctcggaagacgcctatcgagaccacagctgacttgctggactatggtctatgtgtagcaggctcagtcgccgagctattggtctatgtctcttgggcaagtgcaccaagtcaggtccctgccaccatagaagaaagagaagctgtgttagtggcaagccgagagatgggaactgcccttcagttggtgaacattgctagggacattaaaggggacgcaacagaagggagattttacctaccactctcattctttggtcttcgggatgaatcaaagcttgcgatcccgactgattggacggaacctcggcctcaagatttcgacaaactcctcagtctatctccttcgtccacattaccatcttcaaacgcctcagaaagcttccggttcgaatggaagacgtactcgcttccattagtcgcctacgcagaggatcttgccaaacattcttataagggaattgaccgacttcctaccgaggttcaagcgggaatgcgagcggcttgcgcgagctacctactgatcggccgagagatcaaagtcgtttggaaaggagacgtcggagagagaaggacagttgccggatggaggagagtacggaaagtcttgagtgtggtcatgagcggatgggaagggcagtaactcgagtcatgtaattagttatgtcacgcttacattcacgccctccccccacatccgctctaaccgaaaaggaaggagttagacaacctgaagtctaggtccctatttatttttttatagttatgttagtattaagaacgttatttatatttcaaatttttcttttttttctgtacagacgcgtgtacgcatgtaacattatactgaaaaccttgcttgagaaggttttgggacgctcgaaggctttaatttgcggcgcgcggaggccctttcgtcttca

SEQ ID NO: 30 - DNA, 2555 bp, Artificial Sequence
  TEFINtp-crtI-CYC1t
agagaccgggttggcggcgcatttgtgtcccaaaaaacagccccaattgccccaattgaccccaaattgacccagtagcgggcccaaccccggcgagagcccccttctccccacatatcaaacctcccccggttcccacacttgccgttaagggcgtagggtactgcagtctggaatctacgcttgttcagactttgtactagtttctttgtctggccatccgggtaacccatgccggacgcaaaatagactactgaaaatttttttgctttgtggttgggactttagccaagggtataaaagaccaccgtccccgaattacctttcctcttcttttctctctctccttgtcaactcacacccgaaatcgttaagcatttccttctgagtataagaatcattcaaaatggtgagtttcagaggcagcagcaattgccacgggctttgagcacacggccgggtgtggtcccattcccatcgacacaagacgccacgtcatccgaccagcactttttgcagtactaaccgcagggaaaagaacaagatcaggataaacccacagctatcatcgtgggatgtggtatcggtggaatcgccactgccgctcgtcttgctaaagaaggtttccaggtcacggtgttcgagaagaacgactactccggaggtcgatgctctttaatcgagcgagatggttatcgattcgatcaggggcccagtttgctgctcttgccagatctcttcaagcagacattcgaagatttgggagagaagatggaagattgggtcgatctcatcaagtgtgaacccaactatgtttgccacttccacgatgaagagactttcactctttcaaccgacatggcgttgctcaagcgggaagtcgagcgttttgaaggcaaagatggatttgatcggttcttgtcgtttatccaagaagcccacagacattacgagcttgctgtcgttcacgtcctgcagaagaacttccctggcttcgcagcattcttacggctacagttcattggccaaatcctggctcttcaccccttcgagtctatctggacaagagtttgtcgatatttcaagaccgacagattacgaagagtcttctcgtttgcagtgatgtacatgggtcaaagcccatacagtgcgcccggaacatattccttgctccaatacaccgaattgaccgagggcatctggtatccgagaggaggcttttggcaggttcctaatactcttcttcagatcgtcaagcgcaacaatccctcagccaagttcaatttcaacgctccagtttcccaggttcttctctctcctgccaaggaccgagcgactggtgttcgacttgaatccggcgaggaacatcacgccgatgttgtgattgtcaatgctgacctcgtttacgcctccgagcacttgattcctgacgatgccagaaacaagattggccaactgggtgaagtcaagagaagttggtgggctgacttagttggtggaaagaagctcaagggaagttgcagtagtttgagcttctactggagcatggaccgaatcgtggacggtctgggcggacacaatatcttcttggccgaggacttcaagggatcattcgacacaatcttcgaggagttgggtctcccagccgatccttccttttacgtgaacgttccctcgcgaatcgatccttctgccgctcccgaaggcaaagatgctatcgtcattcttgtgccgtgtggccatatcgacgcttcgaaccctcaagattacaacaagcttgttgctcgggcaaggaagtttgtgatccacacgctttccgccaagcttggacttcccgactttgaaaaaatgattgtggcagagaaggttcacgatgctccctcttgggagaaagaattcaacctcaaggacggaagcatcttgggactggctcacaactttatgcaagttcttggtttcaggccgagcaccagacatcccaagtatgacaagttgttctttgtcggggcttcgactcatcccggaactggggttcccatcgtcttggctggagccaagttaactgccaaccaagttctcgaatcctttgaccgatccccagctccagatcccaatatgtcactctccgtaccatatggaaaacctctcaaatcaaatggaacgggtatcgattctcaggtccagctgaagttcatggatttggagagatgggtataccttttggtattgttgattggggccgtgatcgctcgatccgttggtgttcttgctttctgactcgagtcatgtaattagttatgtcacgcttacattcacgccctccccccacatccgctctaaccgaaaaggaaggagttagacaacctgaagtctaggtccctatttatttttttatagttatgttagtattaagaacgttatttatatttcaaatttttcttttttttctgtacagacgcgtgtacgcatgtaacattatactgaaaaccttgcttgagaaggttttgggacgctcgaaggctttaatttgccggccgcgacgagtatctgtctga

SEQ ID NO: 31 - DNA, 1533 bp, Artificial Sequence
  URA3 selection marker
tgcctcctgtctgactcgtcattgccgcctttggagtacgactccaactatgagtgtgcttggatcactttgacgatacattcttcgttggaggctgtgggtctgacagctgcgttttcggcgcggttggccgacaacaatatcagctgcaacgtcattgctggctttcatcatgatcacatttttgtcggcaaaggcgacgcccagagagccattgacgttctttctaatttggaccgatagccgtatagtccagtctatctataagttcaactaactcgtaactattaccataacatatacttcactgccccagataaggttccgataaaaagttctgcagactaaatttatttcagtctcctcttcaccaccaaaatgccctcctacgaagctcgagctaacgtccacaagtccgcctttgccgctcgagtgctcaagctcgtggcagccaagaaaaccaacctgtgtgcttctctggatgttaccaccaccaaggagctcattgagcttgccgataaggtcggaccttatgtgtgcatgatcaagacccatatcgacatcattgacgacttcacctacgccggcactgtgctccccctcaaggaacttgctcttaagcacggtttcttcctgttcgaggacagaaagttcgcagatattggcaacactgtcaagcaccagtacaagaacggtgtctaccgaatcgccgagtggtccgatatcaccaacgcccacggtgtacccggaaccggaatcattgctggcctgcgagctggtgccgaggaaactgtctctgaacagaagaaggaggacgtctctgactacgagaactcccagtacaaggagttcctggtcccctctcccaacgagaagctggccagaggtctgctcatgctggccgagctgtcttgcaagggctctctggccactggcgagtactccaagcagaccattgagcttgcccgatccgaccccgagtttgtggttggcttcattgcccagaaccgacctaagggcgactctgaggactggcttattctgacccccggggtgggtcttgacgacaagggagacgctctcggacagcagtaccgaactgttgaggatgtcatgtctaccggaacggatatcataattgtcggccgaggtctgtacggccagaaccgagatcctattgaggaggccaagcgataccagaaggctggctgggaggcttaccagaagattaactgttagaggttagactatggatatgtcatttaactgtgtatatagagagcgtgcaagtatggagcgcttgttcagcttgtatgatggtcagacgacctgtctgatcgagtatgtatgatactgcacaacctgtgtatccgcatgatctgtccaatggggcatgttgttgtgtttctcgatacggagatgctgggtacaagtagctaatacgattgaactacttatacttatatgaggcttgaagaaagctgacttgtgtatgacttattctcaactacatccccagtcacaataccacca

SEQ ID NO: 32 - DNA, 30 bp, Artificial Sequence
  Primer
gtgcgcttctctcgtctcggtaaccctgtc

SEQ ID NO: 33 - DNA, 44 bp, Artificial Sequence
  Primer
atgcgccgccaacccggtctctggggtgtggtggatggggtgtg

SEQ ID NO: 34 - DNA, 44 bp, Artificial Sequence
  Primer
cacaccccatccaccacaccccagagaccgggttggcggcgcat

SEQ ID NO: 35 - DNA, 39 bp, Artificial Sequence
  Primer
cgccgccaacccggtctcttgaagacgaaagggcctccg

SEQ ID NO: 36 - DNA, 39 bp, Artificial Sequence
  Primer
cggaggccctttcgtcttcaagagaccgggttggcggcg

SEQ ID NO: 37 - DNA, 40 bp, Artificial Sequence
  Primer
gacgagtcagacaggaggcatcagacagatactcgtcgcg

SEQ ID NO: 38 - DNA, 40 bp, Artificial Sequence
  Primer
cgcgacgagtatctgtctgatgcctcctgtctgactcgtc

SEQ ID NO: 39 - DNA, 44 bp, Artificial Sequence
  Primer
atgacgagtcagacaggaggcatggtggtattgtgactggggat

SEQ ID NO: 40 - DNA, 44 bp, Artificial Sequence
  Primer
atccccagtcacaataccaccatgcctcctgtctgactcgtcat

SEQ ID NO: 41 - DNA, 44 bp, Artificial Sequence
  Primer
cggcgtccttctcgtagtccgcttttggtggtgaagaggagact

SEQ ID NO: 42 - DNA, 44 bp, Artificial Sequence
  Primer
agtctcctcttcaccaccaaaagcggactacgagaaggacgccg

SEQ ID NO: 43 - DNA, 30 bp, Artificial Sequence
  Primer
ccactcgtcaccaacagtgccgtgtgttgc

SEQ ID NO: 44 - DNA, 24 bp, Artificial Sequence
  Primer
tcgtacgtctataccaacagatgg

SEQ ID NO: 45 - DNA, 24 bp, Artificial Sequence
  Primer
cgcatacacacacactgccggggg

SEQ ID NO: 46 - DNA, 550 bp, Artificial Sequence
  HMGR native promoter region
tccacacgtcgttcttttttccttagccttttttgcagtgcgcgtgtcccaaaccccagctctacacaccagcacaaacaaagttaagctcagggttgtcgttgaggtcgcttactgtagtcagtgctcgtatggttcgttcaattttcgccaaaaatcgttttgcctttgtatcttgggaataacatcaactgtggttcttcaacaggcctaaggaacgaaacaagccggaccaagatcaggttcaaggtgagtactgagaaggaatagaaggcctaaaggcgcaaaccgacaggtggcaacagctccacaccgaccacgaaggccacgaaatcaaggggtcctaaagttagtctttgtggcctcgacggtcagcgaaaacgcgagaccacaacgcgatcagaaccaggacctaaacaacacaggacggggtcacaataggcttgaacagcaagtacaagctgtgatctctctatatttgattctcaaaccacccctgactacttcagcgcctctgtgacacagcccccctatcatccgactaacacag

SEQ ID NO: 47 - DNA, 30 bp, Artificial Sequence
  Primer
acaatgcctcgaggaggtttaaaagtaact

SEQ ID NO: 48 - DNA, 41 bp, Artificial Sequence
  Primer
gcgccgccaacccggtctctctgtgttagtcggatgatagg

SEQ ID NO: 49 - DNA, 41 bp, Artificial Sequence
  Primer
cctatcatccgactaacacagagagaccgggttggcggcgc

SEQ ID NO: 50 - DNA, 42 bp, Artificial Sequence
  Primer
gacgagtcagacaggaggcactgcggttagtactgcaaaaag

SEQ ID NO: 51 - DNA, 42 bp, Artificial Sequence
  Primer
ctttttgcagtactaaccgcagtgcctcctgtctgactcgtc

SEQ ID NO: 52 - DNA, 44 bp, Artificial Sequence
  Primer
atgcgccgccaacccggtctcttggtggtattgtgactggggat

SEQ ID NO: 53 - DNA, 44 bp, Artificial Sequence
  Primer
atccccagtcacaataccaccaagagaccgggttggcggcgcat

SEQ ID NO: 54 - DNA, 41 bp, Artificial Sequence
  Primer
ctttccaatagctgcttgtagctgcggttagtactgcaaaa

SEQ ID NO: 55 - DNA, 41 bp, Artificial Sequence
  Primer
ttttgcagtactaaccgcagctacaagcagctattggaaag

SEQ ID NO: 56 - DNA, 30 bp, Artificial Sequence
  Primer
gcttaatgtgattgatctcaaacttgatag

SEQ ID NO: 57 - DNA, 24 bp, Artificial Sequence
  Primer
gctgtctctgcgagagcacgtcga

SEQ ID NO: 58 - DNA, 24 bp, Artificial Sequence
  Primer
ggttcgcacaacttctcgggtggc

SEQ ID NO: 59 - DNA, 19 bp, Artificial Sequence
  Primer
ccttgtttagtttggctcc

SEQ ID NO: 60 - DNA, 20 bp, Artificial Sequence
  Primer
aaagccagcaatgacgttgc

SEQ ID NO: 61 - DNA, 40 bp, Artificial Sequence
  Primer
accgtacaactacctcgccaccaaccggggccacaacatc

SEQ ID NO: 62 - DNA, 40 bp, Artificial Sequence
  Primer
gatgttgtggccccggttggtggcgaggtagttgtacggt

SEQ ID NO: 63 - DNA, 40 bp, Artificial Sequence
  Primer
cctgccggcagcccattgtcggtttggagtcccccaaacc

SEQ ID NO: 64 - DNA, 40 bp, Artificial Sequence
  Primer
ggtttgggggactccaaaccgacaatgggctgccggcagg

SEQ ID NO: 65 - DNA, 39 bp, Artificial Sequence
  Primer
gtcttatgatgccgtctccgttttcaccgaggaaatgat

SEQ ID NO: 66 - DNA, 39 bp, Artificial Sequence
  Primer
atcatttcctcggtgaaaacggagacggcatcataagac

SEQ ID NO: 67 - DNA, 40 bp, Artificial Sequence
  Primer
gggtatggatctctactggaaagaaacactcacttgcccc

SEQ ID NO: 68 - DNA, 40 bp, Artificial Sequence
  Primer
ggggcaagtgagtgtttctttccagtagagatccataccc

SEQ ID NO: 69 - DNA, 531 bp, Artificial Sequence
  TEFINt promoter
agagaccgggttggcggcgcatttgtgtcccaaaaaacagccccaattgccccaattgaccccaaattgacccagtagcgggcccaaccccggcgagagcccccttctccccacatatcaaacctcccccggttcccacacttgccgttaagggcgtagggtactgcagtctggaatctacgcttgttcagactttgtactagtttctttgtctggccatccgggtaacccatgccggacgcaaaatagactactgaaaatttttttgctttgtggttgggactttagccaagggtataaaagaccaccgtccccgaattacctttcctcttcttttctctctctccttgtcaactcacacccgaaatcgttaagcatttccttctgagtataagaatcattcaaaatggtgagtttcagaggcagcagcaattgccacgggctttgagcacacggccgggtgtggtcccattcccatcgacacaagacgccacgtcatccgaccagcactttttgcagtactaaccgcag

SEQ ID NO: 70 - DNA, 21 bp, Artificial Sequence
  Primer
atctcttctagatagatgcct

SEQ ID NO: 71 - DNA, 41 bp, Artificial Sequence
  Primer
gcgccgccaacccggtctctgagatttgccacccaacgtcg

SEQ ID NO: 72 - DNA, 41 bp, Artificial Sequence
  Primer
cgacgttgggtggcaaatctcagagaccgggttggcggcgc

SEQ ID NO: 73 - DNA, 42 bp, Artificial Sequence; identical to SEQ ID NO: 50
  Primer

SEQ ID NO: 74 - DNA, 42 bp, Artificial Sequence; identical to SEQ ID NO: 51
  Primer

SEQ ID NO: 75 - DNA, 43 bp, Artificial Sequence
  Primer
gcgccgccaacccggtctcttggtggtattgtgactggggatg

SEQ ID NO: 76 - DNA, 41 bp, Artificial Sequence
  Primer
ttttgcagtactaaccgcaggattataacagcgcggatttc

SEQ ID NO: 77 - DNA, 21 bp, Artificial Sequence
  Primer
taacctggtcaaataccaatg

SEQ ID NO: 78 - DNA, 43 bp, Artificial Sequence
  Primer
catccccagtcacaataccaccaagagaccgggttggcggcgc

SEQ ID NO: 79 - DNA, 41 bp, Artificial Sequence
  Primer
gaaatccgcgctgttataatcctgcggttagtactgcaaaa

SEQ ID NO: 80 - DNA, 21 bp, Artificial Sequence
  Primer
atctcttctagatagatgcct

SEQ ID NO: 81 - DNA, 41 bp, Artificial Sequence; identical to SEQ ID NO: 71
  Primer

SEQ ID NO: 82 - DNA, 41 bp, Artificial Sequence; identical to SEQ ID NO: 72
  Primer

SEQ ID NO: 83 - DNA, 20 bp, Artificial Sequence
  Primer
ctccgatcgctgcgatcaag

SEQ ID NO: 84 - DNA, 20 bp, Artificial Sequence
  Primer
cttgatcgcagcgatcggag

SEQ ID NO: 85 - DNA, 41 bp, Artificial Sequence
  Primer
gacgagtcagacaggaggcataacctggtcaaataccaatg

SEQ ID NO: 86 - DNA, 40 bp, Artificial Sequence
  Primer
cccagtcacaataccaccagattataacagcgcggatttc

SEQ ID NO: 87 - DNA, 40 bp, Artificial Sequence
  Primer
tcaacaattgtaacaacttgtaacctggtcaaataccaat

SEQ ID NO: 88 - DNA, 41 bp, Artificial Sequence
  Primer
cattggtatttgaccaggttatgcctcctgtctgactcgtc

SEQ ID NO: 89 - DNA, 40 bp, Artificial Sequence
  Primer
gaaatccgcgctgttataatctggtggtattgtgactggg

SEQ ID NO: 90 - DNA, 40 bp, Artificial Sequence
  Primer
attggtatttgaccaggttacaagttgttacaattgttga

SEQ ID NO: 91 - DNA, 21 bp, Artificial Sequence
  Primer
tgaaagtcctggaagcagtac